European Patent Specification EP 3 953 709 B1, published November 6, 2024. Title: Diagnostic Reagents. Applicant: The Secretary of State for Environment, Food and Rural Affairs The Penn State Research Foundation. The sequence listing filed with the application follows.

SEQUENCE LISTING (44 sequences)

SEQ ID NO: 1 - protein, 40 aa, Artificial Sequence
  synthetic protein fragment
MTEQQWNFAGIEAAASAIQGNVTSIHSLLDEGKQSLTKLA

SEQ ID NO: 2 - protein, 40 aa, Artificial Sequence
  synthetic protein fragment
NVTSIHSLLDEGKQSLTKLAAAWGGSGSEAYQGVQQKWDA

SEQ ID NO: 3 - protein, 40 aa, Artificial Sequence
  artificial protein fragment
AAWGGSGSEAYQGVQQKWDATATELNNALQNLARTISEAG

SEQ ID NO: 4 - protein, 35 aa, Artificial Sequence
  artificial protein fragment
TATELNNALQNLARTISEAGQAMASTEGNVTGMFA

SEQ ID NO: 5 - protein, 40 aa, Artificial Sequence
  artificial protein fragment
MAEMKTDAATLAQEAGNFERISGDLKTQIDQVESTAGSLQ

SEQ ID NO: 6 - protein, 40 aa, Artificial Sequence
  artificial protein fragment
ISGDLKTQIDQVESTAGSLQGQWRGAAGTAAQAAVVRFQE

SEQ ID NO: 7 - protein, 40 aa, Artificial Sequence
  artificial protein fragment
GQWRGAAGTAAQAAVVRFQEAANKQKQELDEISTNIRQAG

SEQ ID NO: 8 - protein, 40 aa, Artificial Sequence
  artificial protein fragment
AANKQKQELDEISTNIRQAGVQYSRADEEQQQALSSQMGF

SEQ ID NO: 9 - protein, 40 aa, Artificial Sequence
  artificial protein fragment
MTENLTVQPERLGVLASHHDNAAVDASSGVEAAAGLGESV

SEQ ID NO: 10 - protein, 40 aa, Artificial Sequence
  artificial protein fragment
AITHGPYCSQFNDTLNVYLTAHNALGSSLHTAGVDLAKSL

SEQ ID NO: 11 - protein, 40 aa, Artificial Sequence
  artificial protein fragment
AHNALGSSLHTAGVDLAKSLRIAAKIYSEADEAWRKAIDG

SEQ ID NO: 12 - protein, 23 aa, Artificial Sequence
  artificial protein fragment
RIAAKIYSEADEAWRKAIDGLFT

SEQ ID NO: 13 - protein, 16 aa, Artificial Sequence
  artificial protein fragment
MTEQQWNFAGIEAAAS

SEQ ID NO: 14 - protein, 16 aa, Artificial Sequence
  artificial protein fragment
AGIEAAASAIQGNVTS

SEQ ID NO: 15 - protein, 16 aa, Artificial Sequence
  artificial protein fragment
AIQGNVTSIHSLLDEG

SEQ ID NO: 16 - protein, 16 aa, Artificial Sequence
  artificial protein fragment
IHSLLDEGKQSLTKLA

SEQ ID NO: 17 - protein, 16 aa, Artificial Sequence
  artificial protein fragment
KQSLTKLAAAWGGSGS

SEQ ID NO: 18 - protein, 16 aa, Artificial Sequence
  artificial protein fragment
AAWGGSGSEAYQGVQQ

SEQ ID NO: 19 - protein, 16 aa, Artificial Sequence
  artificial protein fragment
EAYQGVQQKWDATATE

SEQ ID NO: 20 - protein, 16 aa, Artificial Sequence
  artificial protein fragment
KWDATATELNNALQNL

SEQ ID NO: 21 - protein, 16 aa, Artificial Sequence
  artificial protein fragment
LNNALQNLARTISEAG

SEQ ID NO: 22 - protein, 16 aa, Artificial Sequence
  artificial protein fragment
ARTISEAGQAMASTEG

SEQ ID NO: 23 - protein, 15 aa, Artificial Sequence
  artificial protein fragment
QAMASTEGNVTGMFA

SEQ ID NO: 24 - protein, 18 aa, Artificial Sequence
  artificial protein fragment
MAEMKTDAATLAQEAGNF

SEQ ID NO: 25 - protein, 16 aa, Artificial Sequence
  artificial protein fragment
QEAGNFERISGDLKTQ

SEQ ID NO: 26 - protein, 18 aa, Artificial Sequence
  artificial protein fragment
ERISGDLKTQIDQVESTA

SEQ ID NO: 27 - protein, 17 aa, Artificial Sequence
  artificial protein fragment
IDQVESTAGSLQGQWRG

SEQ ID NO: 28 - protein, 18 aa, Artificial Sequence
  artificial protein fragment
GSLQGQWRGAAGTAAQAA

SEQ ID NO: 29 - protein, 18 aa, Artificial Sequence
  artificial protein fragment
AGTAAQAAVVRFQEAANK

SEQ ID NO: 30 - protein, 18 aa, Artificial Sequence
  artificial protein fragment
VVRFQEAANKQKQELDEI

SEQ ID NO: 31 - protein, 20 aa, Artificial Sequence
  artificial protein fragment
QKQELDEISTNIRQAGVQYS

SEQ ID NO: 32 - protein, 18 aa, Artificial Sequence
  artificial protein fragment
NIRQAGVQYSRADEEQQQ

SEQ ID NO: 33 - protein, 16 aa, Artificial Sequence
  artificial protein fragment
RADEEQQQALSSQMGF

SEQ ID NO: 34 - protein, 20 aa, Artificial Sequence
  artificial protein fragment
MTENLTVQPERLGVLASHHD

SEQ ID NO: 35 - protein, 20 aa, Artificial Sequence
  artificial protein fragment
PERLGVLASHHDNAAVDASS

SEQ ID NO: 36 - protein, 20 aa, Artificial Sequence
  artificial protein fragment
SHHDNAAVDASSGVEAAAGL

SEQ ID NO: 37 - protein, 20 aa, Artificial Sequence
  artificial protein fragment
DASSGVEAAAGLGESVAITH

SEQ ID NO: 38 - protein, 20 aa, Artificial Sequence
  artificial protein fragment
AAGLGESVAITHGPYCSQFN

SEQ ID NO: 39 - protein, 20 aa, Artificial Sequence
  artificial protein fragment
AITHGPYCSQFNDTLNVYLT

SEQ ID NO: 40 - protein, 20 aa, Artificial Sequence
  artificial protein fragment
SQFNDTLNVYLTAHNALGSS

SEQ ID NO: 41 - protein, 20 aa, Artificial Sequence
  artificial protein fragment
VYLTAHNALGSSLHTAGVDL

SEQ ID NO: 42 - protein, 20 aa, Artificial Sequence
  artificial protein fragment
LGSSLHTAGVDLAKSLRIAA

SEQ ID NO: 43 - protein, 20 aa, Artificial Sequence
  artificial protein fragment
GVDLAKSLRIAAKIYSEADE

SEQ ID NO: 44 - protein, 20 aa, Artificial Sequence
  artificial protein fragment
RIAAKIYSEADEAWRKAIDG